European Patent Specification EP 3 988 660 B1, published May 14, 2025. Title: GENE THERAPY FOR NEURODEGENERATIVE DISORDERS. Applicant: GENZYME CORPORATION. Application Not yet assigned. The sequence listing filed with the application follows.

SEQUENCE LISTING (2 sequences)

SEQ ID NO: 1 - DNA, 885 bp, Homo sapiens
  misc_feature: cDNA sequence of human survival motor neuron (SMN1) gene
atggcgatgagcagcggcggcagtggtggcggcgtcccggagcaggaggattccgtgctgttccggcgcggcacaggccagagcgatgattctgacatttgggatgatacagcactgataaaagcatatgataaagctgtggcttcatttaagcatgctctaaagaatggtgacatttgtgaaacttcgggtaaaccaaaaaccacacctaaaagaaaacctgctaagaagaataaaagccaaaagaagaatactgcagcttccttacaacagtggaaagttggggacaaatgttctgccatttggtcagaagacggttgcatttacccagctaccattgcttcaattgattttaagagagaaacctgtgttgtggtttacactggatatggaaatagagaggagcaaaatctgtccgatctactttccccaatctgtgaagtagctaataatatagaacaaaatgctcaagagaatgaaaatgaaagccaagtttcaacagatgaaagtgagaactccaggtctcctggaaataaatcagataacatcaagcccaaatctgctccatggaactcttttctccctccaccaccccccatgccagggccaagactgggaccaggaaagccaggtctaaaattcaatggcccaccaccgccaccgccaccaccaccaccccacttactatcatgctggctgcctccatttccttctggaccaccaataattcccccaccacctcccatatgtccagattctcttgatgatgctgatgctttgggaagtatgttaatttcatggtacatgagtggctatcatactggctattatatgggtttcagacaaaatcaaaaagaaggaaggtgctcacattccttaaattaa

SEQ ID NO: 2 - protein, 294 aa, Homo sapiens
  misc_feature: amino acid sequence of human survival motor neuron (SMN1) gene
MAMSSGGSGGGVPEQEDSVLFRRGTGQSDDSDIWDDTALIKAYDKAVASFKHALKNGDICETSGKPKTTPKRKPAKKNKSQKKNTAASLQQWKVGDKCSAIWSEDGCIYPATIASIDFKRETCVVVYTGYGNREEQNLSDLLSPICEVANNIEQNAQENENESQVSTDESENSRSPGNKSDNIKPKSAPWNSFLPPPPPMPGPRLGPGKPGLKFNGPPPPPPPPPPHLLSCWLPPFPSGPPIIPPPPPICPDSLDDADALGSMLISWYMSGYHTGYYMGFRQNQKEGRCSHSLN